European Patent Application EP 4 219 734 A1, published August 2, 2023. Title: SYSTEMS AND METHODS OF DIAGNOSING AND CHARACTERIZING INFECTIONS. Applicant: The Translational Genomics Research Institute. The sequence listing filed with the application follows.

SEQUENCE LISTING (431 sequences)

SEQ ID NO: 1 - DNA, 19 bp, synthetic construct
  misc_feature 1..19: note = Primer
  source 1..19: mol_type = other DNA
cgtttcacaactgcggatg

SEQ ID NO: 2 - DNA, 20 bp, synthetic construct
  misc_feature 1..20: note = Primer
  source 1..20: mol_type = other DNA
tggcggtcatgttcttactc

SEQ ID NO: 3 - DNA, 17 bp, synthetic construct
  misc_feature 1..17: note = Primer
  source 1..17: mol_type = other DNA
ttcacaccgccatcgtc

SEQ ID NO: 4 - DNA, 18 bp, synthetic construct
  misc_feature 1..18: note = Primer
  source 1..18: mol_type = other DNA
cagcatctccaccgacag

SEQ ID NO: 5 - DNA, 18 bp, synthetic construct
  misc_feature 1..18: note = Primer
  source 1..18: mol_type = other DNA
cgttcctcaccgtagtgg

SEQ ID NO: 6 - DNA, 19 bp, synthetic construct
  misc_feature 1..19: note = Primer
  source 1..19: mol_type = other DNA
tccagcgtgacataatcgg

SEQ ID NO: 7 - DNA, 21 bp, synthetic construct
  misc_feature 1..21: note = Primer
  source 1..21: mol_type = other DNA
tttccacctacgccgataaag

SEQ ID NO: 8 - DNA, 19 bp, synthetic construct
  misc_feature 1..19: note = Primer
  source 1..19: mol_type = other DNA
ccagcggaataaccaggac

SEQ ID NO: 9 - DNA, 17 bp, synthetic construct
  misc_feature 1..17: note = Primer
  source 1..17: mol_type = other DNA
ggcggcgatgagtttgt

SEQ ID NO: 10 - DNA, 21 bp, synthetic construct
  misc_feature 1..21: note = Primer
  source 1..21: mol_type = other DNA
atgttgcggatagcctgatag

SEQ ID NO: 11 - DNA, 20 bp, synthetic construct
  misc_feature 1..20: note = Primer
  source 1..20: mol_type = other DNA
cgctccactatcaggctatc

SEQ ID NO: 12 - DNA, 20 bp, synthetic construct
  misc_feature 1..20: note = Primer
  source 1..20: mol_type = other DNA
ttcggcgatgggaataaaca

SEQ ID NO: 13 - DNA, 21 bp, synthetic construct
  misc_feature 1..21: note = Primer
  source 1..21: mol_type = other DNA
tgcctatcgccactttattga

SEQ ID NO: 14 - DNA, 19 bp, synthetic construct
  misc_feature 1..19: note = Primer
  source 1..19: mol_type = other DNA
cggtcgttaatcgccttct

SEQ ID NO: 15 - DNA, 19 bp, synthetic construct
  misc_feature 1..19: note = Primer
  source 1..19: mol_type = other DNA
cctcaggtacgctcattcg

SEQ ID NO: 16 - DNA, 19 bp, synthetic construct
  misc_feature 1..19: note = Primer
  source 1..19: mol_type = other DNA
tcgtcacatccctcctctt

SEQ ID NO: 17 - DNA, 20 bp, synthetic construct
  misc_feature 1..20: note = Primer
  source 1..20: mol_type = other DNA
gatcagcagcaaacggtgac

SEQ ID NO: 18 - DNA, 20 bp, synthetic construct
  misc_feature 1..20: note = Primer
  source 1..20: mol_type = other DNA
ggcgatgtaatcctgcgaga

SEQ ID NO: 19 - DNA, 20 bp, synthetic construct
  misc_feature 1..20: note = Primer
  source 1..20: mol_type = other DNA
gggatatccgtggaatgcgt

SEQ ID NO: 20 - DNA, 20 bp, synthetic construct
  misc_feature 1..20: note = Primer
  source 1..20: mol_type = other DNA
taatgtgatcaccgctcccg

SEQ ID NO: 21 - DNA, 20 bp, synthetic construct
  misc_feature 1..20: note = Primer
  source 1..20: mol_type = other DNA
acgagccagcctgatgaaaa

SEQ ID NO: 22 - DNA, 20 bp, synthetic construct
  misc_feature 1..20: note = Primer
  source 1..20: mol_type = other DNA
catcgcaactgctgcatctc

SEQ ID NO: 23 - DNA, 20 bp, synthetic construct
  misc_feature 1..20: note = Primer
  source 1..20: mol_type = other DNA
gccttgcgccttagtttgtt

SEQ ID NO: 24 - DNA, 20 bp, synthetic construct
  misc_feature 1..20: note = Primer
  source 1..20: mol_type = other DNA
ggctatccattttccagccg

SEQ ID NO: 25 - DNA, 20 bp, synthetic construct
  misc_feature 1..20: note = Primer
  source 1..20: mol_type = other DNA
ttcttttccaggagcaacgc

SEQ ID NO: 26 - DNA, 25 bp, synthetic construct
  misc_feature 1..25: note = Primer
  source 1..25: mol_type = other DNA
agcaagacagaaataagtaaaaaga

SEQ ID NO: 27 - DNA, 20 bp, synthetic construct
  misc_feature 1..20: note = Primer
  source 1..20: mol_type = other DNA
tcttcgtcatggtgsgtttc

SEQ ID NO: 28 - DNA, 20 bp, synthetic construct
  misc_feature 1..20: note = Primer
  source 1..20: mol_type = other DNA
aacggaacatggtgagcaac

SEQ ID NO: 29 - DNA, 20 bp, synthetic construct
  misc_feature 1..20: note = Primer
  source 1..20: mol_type = other DNA
gktttgatggctgggtcagt

SEQ ID NO: 30 - DNA, 20 bp, synthetic construct
  misc_feature 1..20: note = Primer
  source 1..20: mol_type = other DNA
tgtttggctttttgcagttg

SEQ ID NO: 31 - DNA, 20 bp, synthetic construct
  misc_feature 1..20: note = Primer
  source 1..20: mol_type = other DNA
tacttrgctttttgcagttg

SEQ ID NO: 32 - DNA, 20 bp, synthetic construct
  misc_feature 1..20: note = Primer
  source 1..20: mol_type = other DNA
tcagtgaaaacracccacga

SEQ ID NO: 33 - DNA, 20 bp, synthetic construct
  misc_feature 1..20: note = Primer
  source 1..20: mol_type = other DNA
atygctgctgtccgagttct

SEQ ID NO: 34 - DNA, 19 bp, synthetic construct
  misc_feature 1..19: note = Primer
  source 1..19: mol_type = other DNA
ccgtcgccgtattactgat

SEQ ID NO: 35 - DNA, 21 bp, synthetic construct
  misc_feature 1..21: note = Primer
  source 1..21: mol_type = other DNA
tctctacaacacgctacccta

SEQ ID NO: 36 - DNA, 21 bp, synthetic construct
  misc_feature 1..21: note = Primer
  source 1..21: mol_type = other DNA
ggtgagaacgatgtgattgtg

SEQ ID NO: 37 - DNA, 18 bp, synthetic construct
  misc_feature 1..18: note = Primer
  source 1..18: mol_type = other DNA
tgacccaaaggcgattcg

SEQ ID NO: 38 - DNA, 18 bp, synthetic construct
  misc_feature 1..18: note = Primer
  source 1..18: mol_type = other DNA
gaagcggttgaggaacag

SEQ ID NO: 39 - DNA, 18 bp, synthetic construct
  misc_feature 1..18: note = Primer
  source 1..18: mol_type = other DNA
acccacgacatgatgtac

SEQ ID NO: 40 - DNA, 20 bp, synthetic construct
  misc_feature 1..20: note = Primer
  source 1..20: mol_type = other DNA
ggacgatccattccataccg

SEQ ID NO: 41 - DNA, 18 bp, synthetic construct
  misc_feature 1..18: note = Primer
  source 1..18: mol_type = other DNA
gacgaagcggtgatccac

SEQ ID NO: 42 - DNA, 21 bp, synthetic construct
  misc_feature 1..21: note = Primer
  source 1..21: mol_type = other DNA
ataggtgtggcttttgtaggg

SEQ ID NO: 43 - DNA, 20 bp, synthetic construct
  misc_feature 1..20: note = Primer
  source 1..20: mol_type = other DNA
ctgctgctaataacgcttgc

SEQ ID NO: 44 - DNA, 26 bp, synthetic construct
  misc_feature 1..26: note = Primer
  source 1..26: mol_type = other DNA
atggttatgaaattgttggtgatgaa

SEQ ID NO: 45 - DNA, 24 bp, synthetic construct
  misc_feature 1..24: note = Primer
  source 1..24: mol_type = other DNA
ccgttgcttgatattctttcgtat

SEQ ID NO: 46 - DNA, 22 bp, synthetic construct
  misc_feature 1..22: note = Primer
  source 1..22: mol_type = other DNA
tacgaaatcagaagtggctcaa

SEQ ID NO: 47 - DNA, 23 bp, synthetic construct
  misc_feature 1..23: note = Primer
  source 1..23: mol_type = other DNA
acgttaaatcctgcattttccaa

SEQ ID NO: 48 - DNA, 23 bp, synthetic construct
  misc_feature 1..23: note = Primer
  source 1..23: mol_type = other DNA
tagcgttggtattaagtggttgt

SEQ ID NO: 49 - DNA, 21 bp, synthetic construct
  misc_feature 1..21: note = Primer
  source 1..21: mol_type = other DNA
gtcatagcatagttcgggtca

SEQ ID NO: 50 - DNA, 19 bp, synthetic construct
  misc_feature 1..19: note = Primer
  source 1..19: mol_type = other DNA
acwggccgtgttgaacgtg

SEQ ID NO: 51 - DNA, 23 bp, synthetic construct
  misc_feature 1..23: note = Primer
  source 1..23: mol_type = other DNA
caccagcttcagcgtagtctaat

SEQ ID NO: 52 - DNA, 24 bp, synthetic construct
  misc_feature 1..24: note = Primer
  source 1..24: mol_type = other DNA
ctcaacwggcatcatgaatggttt

SEQ ID NO: 53 - DNA, 22 bp, synthetic construct
  misc_feature 1..22: note = Primer
  source 1..22: mol_type = other DNA
aggtgacgatgtrcctgtaatc

SEQ ID NO: 54 - DNA, 20 bp, synthetic construct
  misc_feature 1..20: note = Primer
  source 1..20: mol_type = other DNA
cgttgtttgcgaccygtata

SEQ ID NO: 55 - DNA, 22 bp, synthetic construct
  misc_feature 1..22: note = Primer
  source 1..22: mol_type = other DNA
aatgtaaattcgctgrgatcgt

SEQ ID NO: 56 - DNA, 17 bp, synthetic construct
  misc_feature 1..17: note = Primer
  source 1..17: mol_type = other DNA
cgcctggctctgtttca

SEQ ID NO: 57 - DNA, 20 bp, synthetic construct
  misc_feature 1..20: note = Primer
  source 1..20: mol_type = other DNA
agcaagtgcattacgagtct

SEQ ID NO: 58 - DNA, 25 bp, synthetic construct
  misc_feature 1..25: note = Primer
  source 1..25: mol_type = other DNA
gtctgttgaatgatgatgtatgtcg

SEQ ID NO: 59 - DNA, 25 bp, synthetic construct
  misc_feature 1..25: note = Primer
  source 1..25: mol_type = other DNA
atcccattttacaaatggcaaaaca

SEQ ID NO: 60 - DNA, 22 bp, synthetic construct
  misc_feature 1..22: note = Primer
  source 1..22: mol_type = other DNA
tgcagaactagcccattttaca

SEQ ID NO: 61 - DNA, 22 bp, synthetic construct
  misc_feature 1..22: note = Primer
  source 1..22: mol_type = other DNA
tgcwgaactakcccattttaca

SEQ ID NO: 62 - DNA, 24 bp, synthetic construct
  misc_feature 1..24: note = Primer
  source 1..24: mol_type = other DNA
tttagcgracagatttggtttaca

SEQ ID NO: 63 - DNA, 18 bp, synthetic construct
  misc_feature 1..18: note = Primer
  source 1..18: mol_type = other DNA
cggttgccttgctgagtt

SEQ ID NO: 64 - DNA, 21 bp, synthetic construct
  misc_feature 1..21: note = Primer
  source 1..21: mol_type = other DNA
tccgyaaacctcaactcattt

SEQ ID NO: 65 - DNA, 23 bp, synthetic construct
  misc_feature 1..23: note = Primer
  source 1..23: mol_type = other DNA
gccagtgaaccatctaatacagt

SEQ ID NO: 66 - DNA, 24 bp, synthetic construct
  misc_feature 1..24: note = Primer
  source 1..24: mol_type = other DNA
tagagcagcaacaaatcaacaaga

SEQ ID NO: 67 - DNA, 24 bp, synthetic construct
  misc_feature 1..24: note = Primer
  source 1..24: mol_type = other DNA
ttattatgagtcgccttggcaatt

SEQ ID NO: 68 - DNA, 24 bp, synthetic construct
  misc_feature 1..24: note = Primer
  source 1..24: mol_type = other DNA
tagagcagcaacaaatcaacaaga

SEQ ID NO: 69 - DNA, 19 bp, synthetic construct
  misc_feature 1..19: note = Primer
  source 1..19: mol_type = other DNA
tcgcatggcttctgactca

SEQ ID NO: 70 - DNA, 22 bp, synthetic construct
  misc_feature 1..22: note = Primer
  source 1..22: mol_type = other DNA
aaattgcyaaagcacaaggttt

SEQ ID NO: 71 - DNA, 21 bp, synthetic construct
  misc_feature 1..21: note = Primer
  source 1..21: mol_type = other DNA
cgggaattgcytcatggtaag

SEQ ID NO: 72 - DNA, 23 bp, synthetic construct
  misc_feature 1..23: note = Primer
  source 1..23: mol_type = other DNA
gatagcgattactcggttccatc

SEQ ID NO: 73 - DNA, 22 bp, synthetic construct
  misc_feature 1..22: note = Primer
  source 1..22: mol_type = other DNA
cctgtgcctaaaaccagtgaaa

SEQ ID NO: 74 - DNA, 24 bp, synthetic construct
  misc_feature 1..24: note = Primer
  source 1..24: mol_type = other DNA
tcctgatataatcggtgtcacaag

SEQ ID NO: 75 - DNA, 26 bp, synthetic construct
  misc_feature 1..26: note = Primer
  source 1..26: mol_type = other DNA
agaacaagaggtatgtcatctaactt

SEQ ID NO: 76 - DNA, 26 bp, synthetic construct
  misc_feature 1..26: note = Primer
  source 1..26: mol_type = other DNA
ctgatggatatggagacattaaggat

SEQ ID NO: 77 - DNA, 26 bp, synthetic construct
  misc_feature 1..26: note = Primer
  source 1..26: mol_type = other DNA
gtccaattatatgcggatctatacct

SEQ ID NO: 78 - DNA, 26 bp, synthetic construct
  misc_feature 1..26: note = Primer
  source 1..26: mol_type = other DNA
ctgatggatatggagacattaaggat

SEQ ID NO: 79 - DNA, 24 bp, synthetic construct
  misc_feature 1..24: note = Primer
  source 1..24: mol_type = other DNA
aattagttgagtagccatgacagt

SEQ ID NO: 80 - DNA, 23 bp, synthetic construct
  misc_feature 1..23: note = Primer
  source 1..23: mol_type = other DNA
tacggtgtaagtgctgataaagg

SEQ ID NO: 81 - DNA, 25 bp, synthetic construct
  misc_feature 1..25: note = Primer
  source 1..25: mol_type = other DNA
gcttcaaagttaagtccatccaaat

SEQ ID NO: 82 - DNA, 18 bp, synthetic construct
  misc_feature 1..18: note = Primer
  source 1..18: mol_type = other DNA
gccaaccgtggtatgtca

SEQ ID NO: 83 - DNA, 18 bp, synthetic construct
  misc_feature 1..18: note = Primer
  source 1..18: mol_type = other DNA
ttctgccgggtttctttg

SEQ ID NO: 84 - DNA, 18 bp, synthetic construct
  misc_feature 1..18: note = Primer
  source 1..18: mol_type = other DNA
ctcgtgctgctacttctc

SEQ ID NO: 85 - DNA, 22 bp, synthetic construct
  misc_feature 1..22: note = Primer
  source 1..22: mol_type = other DNA
cgtggatgtgctygttaacaac

SEQ ID NO: 86 - DNA, 19 bp, synthetic construct
  misc_feature 1..19: note = Primer
  source 1..19: mol_type = other DNA
aacttrtccttgtgcttgc

SEQ ID NO: 87 - DNA, 21 bp, synthetic construct
  misc_feature 1..21: note = Primer
  source 1..21: mol_type = other DNA
acatagtcgttggcatacaga

SEQ ID NO: 88 - DNA, 23 bp, synthetic construct
  misc_feature 1..23: note = Primer
  source 1..23: mol_type = other DNA
attgttgatgactgttcctcttc

SEQ ID NO: 89 - DNA, 18 bp, synthetic construct
  misc_feature 1..18: note = Primer
  source 1..18: mol_type = other DNA
cgacgaygatgacgaatg

SEQ ID NO: 90 - DNA, 19 bp, synthetic construct
  misc_feature 1..19: note = Primer
  source 1..19: mol_type = other DNA
cgcaattaagtcggtcctg

SEQ ID NO: 91 - DNA, 20 bp, synthetic construct
  misc_feature 1..20: note = Primer
  source 1..20: mol_type = other DNA
ccttcaacgtgratgttcag

SEQ ID NO: 92 - DNA, 19 bp, synthetic construct
  misc_feature 1..19: note = Primer
  source 1..19: mol_type = other DNA
aatwccyacttcgccttca

SEQ ID NO: 93 - DNA, 18 bp, synthetic construct
  misc_feature 1..18: note = Primer
  source 1..18: mol_type = other DNA
tggcgttctggaygtcaa

SEQ ID NO: 94 - DNA, 21 bp, synthetic construct
  misc_feature 1..21: note = Primer
  source 1..21: mol_type = other DNA
agttgtttataccgccaaagc

SEQ ID NO: 95 - DNA, 21 bp, synthetic construct
  misc_feature 1..21: note = Primer
  source 1..21: mol_type = other DNA
agttgtctacactgccaaagc

SEQ ID NO: 96 - DNA, 25 bp, synthetic construct
  misc_feature 1..25: note = Primer
  source 1..25: mol_type = other DNA
acccaaaagtattctgattgttgag

SEQ ID NO: 97 - DNA, 25 bp, synthetic construct
  misc_feature 1..25: note = Primer
  source 1..25: mol_type = other DNA
atgaggtcttattatcggtcaactg

SEQ ID NO: 98 - DNA, 20 bp, synthetic construct
  misc_feature 1..20: note = Primer
  source 1..20: mol_type = other DNA
aatcggcaataccagcagtt

SEQ ID NO: 99 - DNA, 25 bp, synthetic construct
  misc_feature 1..25: note = Primer
  source 1..25: mol_type = other DNA
ccttcacggaataacatatccagat

SEQ ID NO: 100 - DNA, 25 bp, synthetic construct
  misc_feature 1..25: note = Primer
  source 1..25: mol_type = other DNA
gcttattgctaatgactgtgcttat

SEQ ID NO: 101 - DNA, 20 bp, synthetic construct
  misc_feature 1..20: note = Primer
  source 1..20: mol_type = other DNA
tgccgacattgacaaccata

SEQ ID NO: 102 - DNA, 23 bp, synthetic construct
  misc_feature 1..23: note = Primer
  source 1..23: mol_type = other DNA
catctgcttgacctttatgaaac

SEQ ID NO: 103 - DNA, 23 bp, synthetic construct
  misc_feature 1..23: note = Primer
  source 1..23: mol_type = other DNA
gtgaggctaacacatcaaactag

SEQ ID NO: 104 - DNA, 21 bp, synthetic construct
  misc_feature 1..21: note = Primer
  source 1..21: mol_type = other DNA
atgcgggaggtctgtttctac

SEQ ID NO: 105 - DNA, 19 bp, synthetic construct
  misc_feature 1..19: note = Primer
  source 1..19: mol_type = other DNA
ccagccggtaaagaaactc

SEQ ID NO: 106 - DNA, 24 bp, synthetic construct
  misc_feature 1..24: note = Primer
  source 1..24: mol_type = other DNA
gtcaagcaccttaycaccatctag

SEQ ID NO: 107 - DNA, 19 bp, synthetic construct
  misc_feature 1..19: note = Primer
  source 1..19: mol_type = other DNA
ggcatgcttgtgaacaaca

SEQ ID NO: 108 - DNA, 23 bp, synthetic construct
  misc_feature 1..23: note = Primer
  source 1..23: mol_type = other DNA
gtgccrattgaggatctggtttc

SEQ ID NO: 109 - DNA, 22 bp, synthetic construct
  misc_feature 1..22: note = Primer
  source 1..22: mol_type = other DNA
cygttggaccacttcctgtcat

SEQ ID NO: 110 - DNA, 21 bp, synthetic construct
  misc_feature 1..21: note = Primer
  source 1..21: mol_type = other DNA
cgtctagttctgctgtcttgt

SEQ ID NO: 111 - DNA, 18 bp, synthetic construct
  misc_feature 1..18: note = Primer
  source 1..18: mol_type = other DNA
accgtcatgcctgttgtc

SEQ ID NO: 112 - DNA, 23 bp, synthetic construct
  misc_feature 1..23: note = Primer
  source 1..23: mol_type = other DNA
ttgttgattggctaaagggaaac

SEQ ID NO: 113 - DNA, 20 bp, synthetic construct
  misc_feature 1..20: note = Primer
  source 1..20: mol_type = other DNA
cagacgacggcatagtcatt

SEQ ID NO: 114 - DNA, 19 bp, synthetic construct
  misc_feature 1..19: note = Primer
  source 1..19: mol_type = other DNA
ggacaagatgggcggtatg

SEQ ID NO: 115 - DNA, 17 bp, synthetic construct
  misc_feature 1..17: note = Primer
  source 1..17: mol_type = other DNA
cggcgtagtgctcagtg

SEQ ID NO: 116 - DNA, 21 bp, synthetic construct
  misc_feature 1..21: note = Primer
  source 1..21: mol_type = other DNA
caactggatcaagcaggagat

SEQ ID NO: 117 - DNA, 20 bp, synthetic construct
  misc_feature 1..20: note = Primer
  source 1..20: mol_type = other DNA
cgacaacgcattggcataag

SEQ ID NO: 118 - DNA, 22 bp, synthetic construct
  misc_feature 1..22: note = Primer
  source 1..22: mol_type = other DNA
gaattggactgcctctacgatt

SEQ ID NO: 119 - DNA, 18 bp, synthetic construct
  misc_feature 1..18: note = Primer
  source 1..18: mol_type = other DNA
gcacgcccatacagatgt

SEQ ID NO: 120 - DNA, 17 bp, synthetic construct
  misc_feature 1..17: note = Primer
  source 1..17: mol_type = other DNA
aaggcatggaggcgaac

SEQ ID NO: 121 - DNA, 26 bp, synthetic construct
  misc_feature 1..26: note = Primer
  source 1..26: mol_type = other DNA
aagtatataagttctgttccgatggt

SEQ ID NO: 122 - DNA, 24 bp, synthetic construct
  misc_feature 1..24: note = Primer
  source 1..24: mol_type = other DNA
aatactccacactttatccaccaa

SEQ ID NO: 123 - DNA, 20 bp, synthetic construct
  misc_feature 1..20: note = Primer
  source 1..20: mol_type = other DNA
ttcttgcgaacctccttctc

SEQ ID NO: 124 - DNA, 19 bp, synthetic construct
  misc_feature 1..19: note = Primer
  source 1..19: mol_type = other DNA
aacgatgcgacgatccatt

SEQ ID NO: 125 - DNA, 18 bp, synthetic construct
  misc_feature 1..18: note = Primer
  source 1..18: mol_type = other DNA
gcgatttgctgtgcgaaa

SEQ ID NO: 126 - DNA, 21 bp, synthetic construct
  misc_feature 1..21: note = Primer
  source 1..21: mol_type = other DNA
ccgcttgctggtacatatcta

SEQ ID NO: 127 - DNA, 20 bp, synthetic construct
  misc_feature 1..20: note = Primer
  source 1..20: mol_type = other DNA
cctatctcgtccgctatctg

SEQ ID NO: 128 - DNA, 24 bp, synthetic construct
  misc_feature 1..24: note = Primer
  source 1..24: mol_type = other DNA
actattctgcctatcctaattggg

SEQ ID NO: 129 - DNA, 24 bp, synthetic construct
  misc_feature 1..24: note = Primer
  source 1..24: mol_type = other DNA
tcatttaatgttgcgactctttca

SEQ ID NO: 130 - DNA, 28 bp, synthetic construct
  misc_feature 1..28: note = Primer
  source 1..28: mol_type = other DNA
atgactataacaaagcytacaagaaatc

SEQ ID NO: 131 - DNA, 26 bp, synthetic construct
  misc_feature 1..26: note = Primer
  source 1..26: mol_type = other DNA
acaatggtttcataaacagctaagtc

SEQ ID NO: 132 - DNA, 21 bp, synthetic construct
  misc_feature 1..21: note = Primer
  source 1..21: mol_type = other DNA
aacaagccctacaagaaatcc

SEQ ID NO: 133 - DNA, 17 bp, synthetic construct
  misc_feature 1..17: note = Primer
  source 1..17: mol_type = other DNA
cgcacttcggtgtatcg

SEQ ID NO: 134 - DNA, 21 bp, synthetic construct
  misc_feature 1..21: note = Primer
  source 1..21: mol_type = other DNA
aacaagccctacaagaaatcc

SEQ ID NO: 135 - DNA, 17 bp, synthetic construct
  misc_feature 1..17: note = Primer
  source 1..17: mol_type = other DNA
ctcggtgccatcgtagt

SEQ ID NO: 136 - DNA, 20 bp, synthetic construct
  misc_feature 1..20: note = Primer
  source 1..20: mol_type = other DNA
cattgccagatgttcgtgac

SEQ ID NO: 137 - DNA, 20 bp, synthetic construct
  misc_feature 1..20: note = Primer
  source 1..20: mol_type = other DNA
gccatcaacaagcggataac

SEQ ID NO: 138 - DNA, 18 bp, synthetic construct
  misc_feature 1..18: note = Primer
  source 1..18: mol_type = other DNA
aaatctgcccgtgtcgtt

SEQ ID NO: 139 - DNA, 20 bp, synthetic construct
  misc_feature 1..20: note = Primer
  source 1..20: mol_type = other DNA
accatccaccagcatgtaac

SEQ ID NO: 140 - DNA, 23 bp, synthetic construct
  misc_feature 1..23: note = Primer
  source 1..23: mol_type = other DNA
ctcctatctggattatgcgatgt

SEQ ID NO: 141 - DNA, 22 bp, synthetic construct
  misc_feature 1..22: note = Primer
  source 1..22: mol_type = other DNA
cgtcaatagaaccgaagttacc

SEQ ID NO: 142 - DNA, 20 bp, synthetic construct
  misc_feature 1..20: note = Primer
  source 1..20: mol_type = other DNA
caatgactggaacaaagcct

SEQ ID NO: 143 - DNA, 20 bp, synthetic construct
  misc_feature 1..20: note = Primer
  source 1..20: mol_type = other DNA
cgatggaaccaaagttaccc

SEQ ID NO: 144 - DNA, 20 bp, synthetic construct
  misc_feature 1..20: note = Primer
  source 1..20: mol_type = other DNA
ttgtagtgttccaggtcgtc

SEQ ID NO: 145 - DNA, 20 bp, synthetic construct
  misc_feature 1..20: note = Primer
  source 1..20: mol_type = other DNA
ccgtctgctattgttcaagg

SEQ ID NO: 146 - DNA, 20 bp, synthetic construct
  misc_feature 1..20: note = Primer
  source 1..20: mol_type = other DNA
gaaattcaaaaagtccgccc

SEQ ID NO: 147 - DNA, 20 bp, synthetic construct
  misc_feature 1..20: note = Primer
  source 1..20: mol_type = other DNA
ggatagcggtaagagaacgg

SEQ ID NO: 148 - DNA, 20 bp, synthetic construct
  misc_feature 1..20: note = Primer
  source 1..20: mol_type = other DNA
cagcgcgaaattcaaaaagt

SEQ ID NO: 149 - DNA, 20 bp, synthetic construct
  misc_feature 1..20: note = Primer
  source 1..20: mol_type = other DNA
gcgaaagatttgggatcgtc

SEQ ID NO: 150 - DNA, 20 bp, synthetic construct
  misc_feature 1..20: note = Primer
  source 1..20: mol_type = other DNA
gttctcttaccgttatccgc

SEQ ID NO: 151 - DNA, 20 bp, synthetic construct
  misc_feature 1..20: note = Primer
  source 1..20: mol_type = other DNA
tatttcgacaaccgggattc

SEQ ID NO: 152 - DNA, 20 bp, synthetic construct
  misc_feature 1..20: note = Primer
  source 1..20: mol_type = other DNA
tgtgtatgcgatgtctgaac

SEQ ID NO: 153 - DNA, 21 bp, synthetic construct
  misc_feature 1..21: note = Primer
  source 1..21: mol_type = other DNA
atatttcgacaaccgggattc

SEQ ID NO: 154 - DNA, 20 bp, synthetic construct
  misc_feature 1..20: note = Primer
  source 1..20: mol_type = other DNA
gagcgagctaggcttaaaaa

SEQ ID NO: 155 - DNA, 20 bp, synthetic construct
  misc_feature 1..20: note = Primer
  source 1..20: mol_type = other DNA
tcccctgaccttcgattaaa

SEQ ID NO: 156 - DNA, 20 bp, synthetic construct
  misc_feature 1..20: note = Primer
  source 1..20: mol_type = other DNA
gtacgtcattatggaccgtg

SEQ ID NO: 157 - DNA, 20 bp, synthetic construct
  misc_feature 1..20: note = Primer
  source 1..20: mol_type = other DNA
ctataagccgagagtttggc

SEQ ID NO: 158 - DNA, 20 bp, synthetic construct
  misc_feature 1..20: note = Primer
  source 1..20: mol_type = other DNA
tccgtaaaagtgcgaaaaca

SEQ ID NO: 159 - DNA, 20 bp, synthetic construct
  misc_feature 1..20: note = Primer
  source 1..20: mol_type = other DNA
agcttcagtgtaacgcattg

SEQ ID NO: 160 - DNA, 20 bp, synthetic construct
  misc_feature 1..20: note = Primer
  source 1..20: mol_type = other DNA
ccagatgttcgtgatggttt

SEQ ID NO: 161 - DNA, 20 bp, synthetic construct
  misc_feature 1..20: note = Primer
  source 1..20: mol_type = other DNA
cttagcttcagtgtaacgca

SEQ ID NO: 162 - DNA, 20 bp, synthetic construct
  misc_feature 1..20: note = Primer
  source 1..20: mol_type = other DNA
tagagttcagggagtgcgat

SEQ ID NO: 163 - DNA, 23 bp, synthetic construct
  misc_feature 1..23: note = Primer
  source 1..23: mol_type = other DNA
ccgagcagaagtacatcttatgg

SEQ ID NO: 164 - DNA, 20 bp, synthetic construct
  misc_feature 1..20: note = Primer
  source 1..20: mol_type = other DNA
gatttgagygacagccgttt

SEQ ID NO: 165 - DNA, 23 bp, synthetic construct
  misc_feature 1..23: note = Primer
  source 1..23: mol_type = other DNA
gcagaagtacatcttatggctga

SEQ ID NO: 166 - DNA, 24 bp, synthetic construct
  misc_feature 1..24: note = Primer
  source 1..24: mol_type = other DNA
gctaatttctcacaggcaaacttt

SEQ ID NO: 167 - DNA, 22 bp, synthetic construct
  misc_feature 1..22: note = Primer
  source 1..22: mol_type = other DNA
acaacccgtaatgtaagcagag

SEQ ID NO: 168 - DNA, 23 bp, synthetic construct
  misc_feature 1..23: note = Primer
  source 1..23: mol_type = other DNA
gtttgattggtctttggctgatt

SEQ ID NO: 169 - DNA, 21 bp, synthetic construct
  misc_feature 1..21: note = Primer
  source 1..21: mol_type = other DNA
ccatccaacttcactccatct

SEQ ID NO: 170 - DNA, 21 bp, synthetic construct
  misc_feature 1..21: note = Primer
  source 1..21: mol_type = other DNA
cgacaggaatagcttggaagg

SEQ ID NO: 171 - DNA, 21 bp, synthetic construct
  misc_feature 1..21: note = Primer
  source 1..21: mol_type = other DNA
ccagttatcacagtgccattc

SEQ ID NO: 172 - DNA, 20 bp, synthetic construct
  misc_feature 1..20: note = Primer
  source 1..20: mol_type = other DNA
caatttatgccacgccgaac

SEQ ID NO: 173 - DNA, 20 bp, synthetic construct
  misc_feature 1..20: note = Primer
  source 1..20: mol_type = other DNA
taatttatgtcacgccgaac

SEQ ID NO: 174 - DNA, 24 bp, synthetic construct
  misc_feature 1..24: note = Primer
  source 1..24: mol_type = other DNA
gataaacaacaatacccagtgctt

SEQ ID NO: 175 - DNA, 21 bp, synthetic construct
  misc_feature 1..21: note = Primer
  source 1..21: mol_type = other DNA
gtgctaacttgcgtgatacga

SEQ ID NO: 176 - DNA, 26 bp, synthetic construct
  misc_feature 1..26: note = Primer
  source 1..26: mol_type = other DNA
tccatattggcataggaaagattaca

SEQ ID NO: 177 - DNA, 26 bp, synthetic construct
  misc_feature 1..26: note = Primer
  source 1..26: mol_type = other DNA
tccatattggcataagacaggttaca

SEQ ID NO: 178 - DNA, 21 bp, synthetic construct
  misc_feature 1..21: note = Primer
  source 1..21: mol_type = other DNA
gacgttcagtggttcrgatct

SEQ ID NO: 179 - DNA, 18 bp, synthetic construct
  misc_feature 1..18: note = Primer
  source 1..18: mol_type = other DNA
kgctcgccagtcgaaagt

SEQ ID NO: 180 - DNA, 22 bp, synthetic construct
  misc_feature 1..22: note = Primer
  source 1..22: mol_type = other DNA
cgacgttcagtggttcrgatct

SEQ ID NO: 181 - DNA, 18 bp, synthetic construct
  misc_feature 1..18: note = Primer
  source 1..18: mol_type = other DNA
gckgctcgccagtcgaaa

SEQ ID NO: 182 - DNA, 23 bp, synthetic construct
  misc_feature 1..23: note = Primer
  source 1..23: mol_type = other DNA
accaatctaagctacgccaactt

SEQ ID NO: 183 - DNA, 19 bp, synthetic construct
  misc_feature 1..19: note = Primer
  source 1..19: mol_type = other DNA
cctgagttcccatccagcg

SEQ ID NO: 184 - DNA, 22 bp, synthetic construct
  misc_feature 1..22: note = Primer
  source 1..22: mol_type = other DNA
tacgcactgtgatttgaccaat

SEQ ID NO: 185 - DNA, 20 bp, synthetic construct
  misc_feature 1..20: note = Primer
  source 1..20: mol_type = other DNA
ggakcaacgatgcctggtag

SEQ ID NO: 186 - DNA, 24 bp, synthetic construct
  misc_feature 1..24: note = Primer
  source 1..24: mol_type = other DNA
cgcatatatcaccaataccaactt

SEQ ID NO: 187 - DNA, 20 bp, synthetic construct
  misc_feature 1..20: note = Primer
  source 1..20: mol_type = other DNA
gttccaggakcaacgatgcc

SEQ ID NO: 188 - DNA, 19 bp, synthetic construct
  misc_feature 1..19: note = Primer
  source 1..19: mol_type = other DNA
ccgtcacgctgttgttagg

SEQ ID NO: 189 - DNA, 21 bp, synthetic construct
  misc_feature 1..21: note = Primer
  source 1..21: mol_type = other DNA
cgctcatcagcacgataaagt

SEQ ID NO: 190 - DNA, 23 bp, synthetic construct
  misc_feature 1..23: note = Primer
  source 1..23: mol_type = other DNA
cgctgattctggtcatttacttc

SEQ ID NO: 191 - DNA, 19 bp, synthetic construct
  misc_feature 1..19: note = Primer
  source 1..19: mol_type = other DNA
acggctttctgccttaggt

SEQ ID NO: 192 - DNA, 19 bp, synthetic construct
  misc_feature 1..19: note = Primer
  source 1..19: mol_type = other DNA
cgatgtgcagcaccagtaa

SEQ ID NO: 193 - DNA, 21 bp, synthetic construct
  misc_feature 1..21: note = Primer
  source 1..21: mol_type = other DNA
tcggttcgctttcacttttct

SEQ ID NO: 194 - DNA, 19 bp, synthetic construct
  misc_feature 1..19: note = Primer
  source 1..19: mol_type = other DNA
gacgatgtcactggctgag

SEQ ID NO: 195 - DNA, 18 bp, synthetic construct
  misc_feature 1..18: note = Primer
  source 1..18: mol_type = other DNA
ccacaacccaggaagcag

SEQ ID NO: 196 - DNA, 18 bp, synthetic construct
  misc_feature 1..18: note = Primer
  source 1..18: mol_type = other DNA
tggcgcagaccctgaaaa

SEQ ID NO: 197 - DNA, 21 bp, synthetic construct
  misc_feature 1..21: note = Primer
  source 1..21: mol_type = other DNA
atatcgttggtggtgccataa

SEQ ID NO: 198 - DNA, 18 bp, synthetic construct
  misc_feature 1..18: note = Primer
  source 1..18: mol_type = other DNA
atggcgcagaccctgaaa

SEQ ID NO: 199 - DNA, 18 bp, synthetic construct
  misc_feature 1..18: note = Primer
  source 1..18: mol_type = other DNA
ccgctgccggttttatcg

SEQ ID NO: 200 - DNA, 18 bp, synthetic construct
  misc_feature 1..18: note = Primer
  source 1..18: mol_type = other DNA
gagccgacgctcaacacc

SEQ ID NO: 201 - DNA, 18 bp, synthetic construct
  misc_feature 1..18: note = Primer
  source 1..18: mol_type = other DNA
cccgacaacccacgatgt

SEQ ID NO: 202 - DNA, 18 bp, synthetic construct
  misc_feature 1..18: note = Primer
  source 1..18: mol_type = other DNA
gctcaacaccgcgatccc

SEQ ID NO: 203 - DNA, 18 bp, synthetic construct
  misc_feature 1..18: note = Primer
  source 1..18: mol_type = other DNA
cccgacaacccacgatgt

SEQ ID NO: 204 - DNA, 19 bp, synthetic construct
  misc_feature 1..19: note = Primer
  source 1..19: mol_type = other DNA
ttcgtctggatcgcactga

SEQ ID NO: 205 - DNA, 20 bp, synthetic construct
  misc_feature 1..20: note = Primer
  source 1..20: mol_type = other DNA
gatgattctcgccgctgaag

SEQ ID NO: 206 - DNA, 19 bp, synthetic construct
  misc_feature 1..19: note = Primer
  source 1..19: mol_type = other DNA
cgctggttctggtgaccta

SEQ ID NO: 207 - DNA, 20 bp, synthetic construct
  misc_feature 1..20: note = Primer
  source 1..20: mol_type = other DNA
gatgattctcgccgctgaag

SEQ ID NO: 208 - DNA, 19 bp, synthetic construct
  misc_feature 1..19: note = Primer
  source 1..19: mol_type = other DNA
aatggctgttggttggacg

SEQ ID NO: 209 - DNA, 23 bp, synthetic construct
  misc_feature 1..23: note = Primer
  source 1..23: mol_type = other DNA
catactttcggttgggtaatgct

SEQ ID NO: 210 - DNA, 23 bp, synthetic construct
  misc_feature 1..23: note = Primer
  source 1..23: mol_type = other DNA
aatatgccgttgtaactcgttca

SEQ ID NO: 211 - DNA, 24 bp, synthetic construct
  misc_feature 1..24: note = Primer
  source 1..24: mol_type = other DNA
acacaatcacatgatccgttatcg

SEQ ID NO: 212 - DNA, 24 bp, synthetic construct
  misc_feature 1..24: note = Primer
  source 1..24: mol_type = other DNA
agtatgcagttgtaactcgctcta

SEQ ID NO: 213 - DNA, 22 bp, synthetic construct
  misc_feature 1..22: note = Primer
  source 1..22: mol_type = other DNA
caccaccaccagaaacgataac

SEQ ID NO: 214 - DNA, 18 bp, synthetic construct
  misc_feature 1..18: note = Primer
  source 1..18: mol_type = other DNA
gtgattggttgcggtcca

SEQ ID NO: 215 - DNA, 18 bp, synthetic construct
  misc_feature 1..18: note = Primer
  source 1..18: mol_type = other DNA
cccgccaccagacactat

SEQ ID NO: 216 - DNA, 22 bp, synthetic construct
  misc_feature 1..22: note = Primer
  source 1..22: mol_type = other DNA
ygagaatggagtaattggctct

SEQ ID NO: 217 - DNA, 24 bp, synthetic construct
  misc_feature 1..24: note = Primer
  source 1..24: mol_type = other DNA
watttcaccaccaccagaaacaaa

SEQ ID NO: 218 - DNA, 18 bp, synthetic construct
  misc_feature 1..18: note = Primer
  source 1..18: mol_type = other DNA
gggwgccaatcgggttat

SEQ ID NO: 219 - DNA, 18 bp, synthetic construct
  misc_feature 1..18: note = Primer
  source 1..18: mol_type = other DNA
ctcagtgagtctgcgaaa

SEQ ID NO: 220 - DNA, 18 bp, synthetic construct
  misc_feature 1..18: note = Primer
  source 1..18: mol_type = other DNA
ctcggtgagcctgcgaaa

SEQ ID NO: 221 - DNA, 21 bp, synthetic construct
  misc_feature 1..21: note = Primer
  source 1..21: mol_type = other DNA
aaagactacgagcagaatggc

SEQ ID NO: 222 - DNA, 24 bp, synthetic construct
  misc_feature 1..24: note = Primer
  source 1..24: mol_type = other DNA
acggtaagtgaagtaagtgtgaag

SEQ ID NO: 223 - DNA, 19 bp, synthetic construct
  misc_feature 1..19: note = Primer
  source 1..19: mol_type = other DNA
aacgctgccattgttacca

SEQ ID NO: 224 - DNA, 21 bp, synthetic construct
  misc_feature 1..21: note = Primer
  source 1..21: mol_type = other DNA
aagccttgaagtgttctggag

SEQ ID NO: 225 - DNA, 23 bp, synthetic construct
  misc_feature 1..23: note = Primer
  source 1..23: mol_type = other DNA
aagacaggaggtatcggatttga

SEQ ID NO: 226 - DNA, 22 bp, synthetic construct
  misc_feature 1..22: note = Primer
  source 1..22: mol_type = other DNA
cgtaggcagctaagttctcgta

SEQ ID NO: 227 - DNA, 23 bp, synthetic construct
  misc_feature 1..23: note = Primer
  source 1..23: mol_type = other DNA
aagaccgcatcaatatcgtcatc

SEQ ID NO: 228 - DNA, 20 bp, synthetic construct
  misc_feature 1..20: note = Primer
  source 1..20: mol_type = other DNA
catagcaagccgtccaagaa

SEQ ID NO: 229 - DNA, 24 bp, synthetic construct
  misc_feature 1..24: note = Primer
  source 1..24: mol_type = other DNA
aagactcttacgaaccatgttgtt

SEQ ID NO: 230 - DNA, 21 bp, synthetic construct
  misc_feature 1..21: note = Primer
  source 1..21: mol_type = other DNA
cctctggctcggaatctattg

SEQ ID NO: 231 - DNA, 23 bp, synthetic construct
  misc_feature 1..23: note = Primer
  source 1..23: mol_type = other DNA
aagcactgacctataaccaatgg

SEQ ID NO: 232 - DNA, 22 bp, synthetic construct
  misc_feature 1..22: note = Primer
  source 1..22: mol_type = other DNA
cccaggaatgttcggaaagaaa

SEQ ID NO: 233 - DNA, 22 bp, synthetic construct
  misc_feature 1..22: note = Primer
  source 1..22: mol_type = other DNA
aagcattcagagacacaaccaa

SEQ ID NO: 234 - DNA, 21 bp, synthetic construct
  misc_feature 1..21: note = Primer
  source 1..21: mol_type = other DNA
aaccaacaccaccaatgacat

SEQ ID NO: 235 - DNA, 24 bp, synthetic construct
  misc_feature 1..24: note = Primer
  source 1..24: mol_type = other DNA
aaggtgagcagctaatctttaagg

SEQ ID NO: 236 - DNA, 24 bp, synthetic construct
  misc_feature 1..24: note = Primer
  source 1..24: mol_type = other DNA
tgaccctgaaattccattctttga

SEQ ID NO: 237 - DNA, 22 bp, synthetic construct
  misc_feature 1..22: note = Primer
  source 1..22: mol_type = other DNA
aagtcgcacaacatcttgaagg

SEQ ID NO: 238 - DNA, 24 bp, synthetic construct
  misc_feature 1..24: note = Primer
  source 1..24: mol_type = other DNA
agatttgagcaccaccaataatga

SEQ ID NO: 239 - DNA, 24 bp, synthetic construct
  misc_feature 1..24: note = Primer
  source 1..24: mol_type = other DNA
aatcaatatcacgacagcgatcaa

SEQ ID NO: 240 - DNA, 19 bp, synthetic construct
  misc_feature 1..19: note = Pirmer
  source 1..19: mol_type = other DNA
cttcacgggatgggtctca

SEQ ID NO: 241 - DNA, 20 bp, synthetic construct
  misc_feature 1..20: note = Primer
  source 1..20: mol_type = other DNA
aatcagtggctccttgttgg

SEQ ID NO: 242 - DNA, 24 bp, synthetic construct
  misc_feature 1..24: note = Primer
  source 1..24: mol_type = other DNA
ggaagaacacccatagagtcaaat

SEQ ID NO: 243 - DNA, 20 bp, synthetic construct
  misc_feature 1..20: note = Primer
  source 1..20: mol_type = other DNA
aatcagtggcttcttgtcgg

SEQ ID NO: 244 - DNA, 24 bp, synthetic construct
  misc_feature 1..24: note = Primer
  source 1..24: mol_type = other DNA
gtggatgatagataagtggatggt

SEQ ID NO: 245 - DNA, 20 bp, synthetic construct
  misc_feature 1..20: note = Primer
  source 1..20: mol_type = other DNA
aatggcgtaatcggtagtgg

SEQ ID NO: 246 - DNA, 23 bp, synthetic construct
  misc_feature 1..23: note = Primer
  source 1..23: mol_type = other DNA
gcttgaaattccgttctttgaca

SEQ ID NO: 247 - DNA, 19 bp, synthetic construct
  misc_feature 1..19: note = Primer
  source 1..19: mol_type = other DNA
acgcattgctgtcattggt

SEQ ID NO: 248 - DNA, 18 bp, synthetic construct
  misc_feature 1..18: note = Primer
  source 1..18: mol_type = other DNA
ctcgctggcactggaatc

SEQ ID NO: 249 - DNA, 19 bp, synthetic construct
  misc_feature 1..19: note = Primer
  source 1..19: mol_type = other DNA
actctatgccgaggctctg

SEQ ID NO: 250 - DNA, 20 bp, synthetic construct
  misc_feature 1..20: note = Primer
  source 1..20: mol_type = other DNA
cgctgacgactcaaggtaac

SEQ ID NO: 251 - DNA, 18 bp, synthetic construct
  misc_feature 1..18: note = Primer
  source 1..18: mol_type = other DNA
watgggagatcgcgtgcg

SEQ ID NO: 252 - DNA, 20 bp, synthetic construct
  misc_feature 1..20: note = Primer
  source 1..20: mol_type = other DNA
gcwgtaccacccgacaatct

SEQ ID NO: 253 - DNA, 18 bp, synthetic construct
  misc_feature 1..18: note = Primer
  source 1..18: mol_type = other DNA
gcagggtcaagtygtcgg

SEQ ID NO: 254 - DNA, 18 bp, synthetic construct
  misc_feature 1..18: note = Primer
  source 1..18: mol_type = other DNA
tcggactcgacsgcatag

SEQ ID NO: 255 - DNA, 18 bp, synthetic construct
  misc_feature 1..18: note = Primer
  source 1..18: mol_type = other DNA
acccgacaacttgaccct

SEQ ID NO: 256 - DNA, 21 bp, synthetic construct
  misc_feature 1..21: note = Primer
  source 1..21: mol_type = other DNA
accaacacaacaatggagtca

SEQ ID NO: 257 - DNA, 19 bp, synthetic construct
  misc_feature 1..19: note = Primer
  source 1..19: mol_type = other DNA
aatctcacccaggctcagt

SEQ ID NO: 258 - DNA, 18 bp, synthetic construct
  misc_feature 1..18: note = Primer
  source 1..18: mol_type = other DNA
ccgttcaagcgcagtcat

SEQ ID NO: 259 - DNA, 20 bp, synthetic construct
  misc_feature 1..20: note = Primer
  source 1..20: mol_type = other DNA
gctggtggttatgcactcag

SEQ ID NO: 260 - DNA, 19 bp, synthetic construct
  misc_feature 1..19: note = Primer
  source 1..19: mol_type = other DNA
cgcccaagaaggatttccg

SEQ ID NO: 261 - DNA, 19 bp, synthetic construct
  misc_feature 1..19: note = Primer
  source 1..19: mol_type = other DNA
cgtgctgtcgaaccttcaa

SEQ ID NO: 262 - DNA, 21 bp, synthetic construct
  misc_feature 1..21: note = Primer
  source 1..21: mol_type = other DNA
gctggacccagatcctttaca

SEQ ID NO: 263 - DNA, 22 bp, synthetic construct
  misc_feature 1..22: note = Primer
  source 1..22: mol_type = other DNA
catcattttcggcatcgtcaac

SEQ ID NO: 264 - DNA, 18 bp, synthetic construct
  misc_feature 1..18: note = Primer
  source 1..18: mol_type = other DNA
gcgacaaggcataggctt

SEQ ID NO: 265 - DNA, 22 bp, synthetic construct
  misc_feature 1..22: note = Primer
  source 1..22: mol_type = other DNA
gtcaacataacctcggacagtt

SEQ ID NO: 266 - DNA, 18 bp, synthetic construct
  misc_feature 1..18: note = Primer
  source 1..18: mol_type = other DNA
ctcggccatcagcttacg

SEQ ID NO: 267 - DNA, 24 bp, synthetic construct
  misc_feature 1..24: note = Primer
  source 1..24: mol_type = other DNA
aaagccttaatgacaggtttgagt

SEQ ID NO: 268 - DNA, 24 bp, synthetic construct
  misc_feature 1..24: note = Primer
  source 1..24: mol_type = other DNA
gaagatggagcagatgtgattgat

SEQ ID NO: 269 - DNA, 23 bp, synthetic construct
  misc_feature 1..23: note = Primer
  source 1..23: mol_type = other DNA
ggcaaagtcagattgcaaacttg

SEQ ID NO: 270 - DNA, 22 bp, synthetic construct
  misc_feature 1..22: note = Primer
  source 1..22: mol_type = other DNA
cctcttccggattcgtttcaac

SEQ ID NO: 271 - DNA, 23 bp, synthetic construct
  misc_feature 1..23: note = Primer
  source 1..23: mol_type = other DNA
ccaggtcctaatgctgatagacg

SEQ ID NO: 272 - DNA, 24 bp, synthetic construct
  misc_feature 1..24: note = Primer
  source 1..24: mol_type = other DNA
accgtcgtttacgttctgtaggtg

SEQ ID NO: 273 - DNA, 23 bp, synthetic construct
  misc_feature 1..23: note = Primer
  source 1..23: mol_type = other DNA
ccaggtcctaatgctgatagacg

SEQ ID NO: 274 - DNA, 22 bp, synthetic construct
  misc_feature 1..22: note = Primer
  source 1..22: mol_type = other DNA
ggaccaagcaaayccattagct

SEQ ID NO: 275 - DNA, 21 bp, synthetic construct
  misc_feature 1..21: note = Primer
  source 1..21: mol_type = other DNA
gtgaaggcatccaatsaactt

SEQ ID NO: 276 - DNA, 24 bp, synthetic construct
  misc_feature 1..24: note = Primer
  source 1..24: mol_type = other DNA
aaacmacaaagagaacacagagat

SEQ ID NO: 277 - DNA, 24 bp, synthetic construct
  misc_feature 1..24: note = Primer
  source 1..24: mol_type = other DNA
ggaacgatgcctatctcatatgct

SEQ ID NO: 278 - DNA, 25 bp, synthetic construct
  misc_feature 1..25: note = Primer
  source 1..25: mol_type = other DNA
atagcgtcattattccaggaatgca

SEQ ID NO: 279 - DNA, 19 bp, synthetic construct
  misc_feature 1..19: note = Primer
  source 1..19: mol_type = other DNA
cggctcgacttcctgatga

SEQ ID NO: 280 - DNA, 20 bp, synthetic construct
  misc_feature 1..20: note = Primer
  source 1..20: mol_type = other DNA
tgtgcggtattgggaaacag

SEQ ID NO: 281 - DNA, 25 bp, synthetic construct
  misc_feature 1..25: note = Primer
  source 1..25: mol_type = other DNA
gccacactatcataaccactaccga

SEQ ID NO: 282 - DNA, 25 bp, synthetic construct
  misc_feature 1..25: note = Primer
  source 1..25: mol_type = other DNA
tccaagagcaataagggcataccaa

SEQ ID NO: 283 - DNA, 20 bp, synthetic construct
  misc_feature 1..20: note = Primer
  source 1..20: mol_type = other DNA
acactcttggcggtttcact

SEQ ID NO: 284 - DNA, 24 bp, synthetic construct
  misc_feature 1..24: note = Primer
  source 1..24: mol_type = other DNA
cctaagggccaatctgaacctatt

SEQ ID NO: 285 - DNA, 27 bp, synthetic construct
  misc_feature 1..27: note = Primer
  source 1..27: mol_type = other DNA
caaccattgatttcaaagaaggactac

SEQ ID NO: 286 - DNA, 21 bp, synthetic construct
  misc_feature 1..21: note = Primer
  source 1..21: mol_type = other DNA
tcaaagcctgtcggaattggt

SEQ ID NO: 287 - DNA, 28 bp, synthetic construct
  misc_feature 1..28: note = Primer
  source 1..28: mol_type = other DNA
atttaatcgtggaatacgagtttgctaa

SEQ ID NO: 288 - DNA, 24 bp, synthetic construct
  misc_feature 1..24: note = Primer
  source 1..24: mol_type = other DNA
cgtcaattcctgcatgttttaagg

SEQ ID NO: 289 - DNA, 24 bp, synthetic construct
  misc_feature 1..24: note = Primer
  source 1..24: mol_type = other DNA
agtttgagctgtcttggttcattg

SEQ ID NO: 290 - DNA, 24 bp, synthetic construct
  misc_feature 1..24: note = Primer
  source 1..24: mol_type = other DNA
tgcagcagatcctactccttgtac

SEQ ID NO: 291 - DNA, 25 bp, synthetic construct
  misc_feature 1..25: note = Primer
  source 1..25: mol_type = other DNA
ctttctgggcttccattggtttatc

SEQ ID NO: 292 - DNA, 22 bp, synthetic construct
  misc_feature 1..22: note = Primer
  source 1..22: mol_type = other DNA
cgagctctcatactgcattcca

SEQ ID NO: 293 - DNA, 26 bp, synthetic construct
  misc_feature 1..26: note = Primer
  source 1..26: mol_type = other DNA
cttcttccaaatgttccattcttttt

SEQ ID NO: 294 - DNA, 24 bp, synthetic construct
  misc_feature 1..24: note = Primer
  source 1..24: mol_type = other DNA
accagatcgtttaagtgcatcaaa

SEQ ID NO: 295 - DNA, 20 bp, synthetic construct
  misc_feature 1..20: note = Primer
  source 1..20: mol_type = other DNA
aacgaagggcaggtagaagc

SEQ ID NO: 296 - DNA, 20 bp, synthetic construct
  misc_feature 1..20: note = Primer
  source 1..20: mol_type = other DNA
tgaccacaagcagcgtcaat

SEQ ID NO: 297 - DNA, 21 bp, synthetic construct
  misc_feature 1..21: note = Primer
  source 1..21: mol_type = other DNA
gtgaggaacgcagcaaattga

SEQ ID NO: 298 - DNA, 20 bp, synthetic construct
  misc_feature 1..20: note = Primer
  source 1..20: mol_type = other DNA
gcttctacctgcccttcgtt

SEQ ID NO: 299 - DNA, 19 bp, synthetic construct
  misc_feature 1..19: note = Primer
  source 1..19: mol_type = other DNA
ggatcaaacggcctgcaca

SEQ ID NO: 300 - DNA, 22 bp, synthetic construct
  misc_feature 1..22: note = Primer
  source 1..22: mol_type = other DNA
tggctccaatggtytacaccaa

SEQ ID NO: 301 - DNA, 29 bp, synthetic construct
  misc_feature 1..29: note = Primer
  source 1..29: mol_type = other DNA
gtcaaaaatcatgaacctcattacttatg

SEQ ID NO: 302 - DNA, 29 bp, synthetic construct
  misc_feature 1..29: note = Primer
  source 1..29: mol_type = other DNA
atttcatatatgtaattcctccacatctc

SEQ ID NO: 303 - DNA, 29 bp, synthetic construct
  misc_feature 1..29: note = Primer
  source 1..29: mol_type = other DNA
caaatattatctcgtaatttaccttgttc

SEQ ID NO: 304 - DNA, 29 bp, synthetic construct
  misc_feature 1..29: note = Primer
  source 1..29: mol_type = other DNA
ctctgctttatattataaaattacggctg

SEQ ID NO: 305 - DNA, 27 bp, synthetic construct
  misc_feature 1..27: note = Primer
  source 1..27: mol_type = other DNA
cactttttattcttcaaagatttgagc

SEQ ID NO: 306 - DNA, 21 bp, synthetic construct
  misc_feature 1..21: note = Primer
  source 1..21: mol_type = other DNA
ctcatgttacaratacttgcg

SEQ ID NO: 307 - DNA, 21 bp, synthetic construct
  misc_feature 1..21: note = Primer
  source 1..21: mol_type = other DNA
ccttgataatagccttcttgg

SEQ ID NO: 308 - DNA, 26 bp, synthetic construct
  misc_feature 1..26: note = Primer
  source 1..26: mol_type = other DNA
cgttataagtgtacgaatggtttttg

SEQ ID NO: 309 - DNA, 21 bp, synthetic construct
  misc_feature 1..21: note = Primer
  source 1..21: mol_type = other DNA
tcatctgcagaatgggaagtt

SEQ ID NO: 310 - DNA, 20 bp, synthetic construct
  misc_feature 1..20: note = Primer
  source 1..20: mol_type = other DNA
gaagctttgggcgataaaga

SEQ ID NO: 311 - DNA, 23 bp, synthetic construct
  misc_feature 1..23: note = Primer
  source 1..23: mol_type = other DNA
gcactgtctcgtttagaccaatc

SEQ ID NO: 312 - DNA, 24 bp, synthetic construct
  misc_feature 1..24: note = Primer
  source 1..24: mol_type = other DNA
tccagtctataaaggstatgtcag

SEQ ID NO: 313 - DNA, 24 bp, synthetic construct
  misc_feature 1..24: note = Primer
  source 1..24: mol_type = other DNA
acttataatggcttcatgcttacc

SEQ ID NO: 314 - DNA, 22 bp, synthetic construct
  misc_feature 1..22: note = Primer
  source 1..22: mol_type = other DNA
accacaaacacacttaaagatg

SEQ ID NO: 315 - DNA, 25 bp, synthetic construct
  misc_feature 1..25: note = Primer
  source 1..25: mol_type = other DNA
caatttcaagtatttggtccataac

SEQ ID NO: 316 - DNA, 22 bp, synthetic construct
  misc_feature 1..22: note = Primer
  source 1..22: mol_type = other DNA
aacacaacgaacacattgaaag

SEQ ID NO: 317 - DNA, 22 bp, synthetic construct
  misc_feature 1..22: note = Primer
  source 1..22: mol_type = other DNA
cgtatttctcaatcacatcagc

SEQ ID NO: 318 - DNA, 24 bp, synthetic construct
  misc_feature 1..24: note = Primer
  source 1..24: mol_type = other DNA
cgaagtatagacactggagcgata

SEQ ID NO: 319 - DNA, 19 bp, synthetic construct
  misc_feature 1..19: note = Primer
  source 1..19: mol_type = other DNA
gcgactctcttggcgttta

SEQ ID NO: 320 - DNA, 22 bp, synthetic construct
  misc_feature 1..22: note = Primer
  source 1..22: mol_type = other DNA
tcagttcattgctcacgatatg

SEQ ID NO: 321 - DNA, 20 bp, synthetic construct
  misc_feature 1..20: note = Primer
  source 1..20: mol_type = other DNA
gccaacggctacagtgataa

SEQ ID NO: 322 - DNA, 24 bp, synthetic construct
  misc_feature 1..24: note = Primer
  source 1..24: mol_type = other DNA
caggatatttttcaaactccttca

SEQ ID NO: 323 - DNA, 20 bp, synthetic construct
  misc_feature 1..20: note = Primer
  source 1..20: mol_type = other DNA
tggaggaccaaggatattcg

SEQ ID NO: 324 - DNA, 27 bp, synthetic construct
  misc_feature 1..27: note = Primer
  source 1..27: mol_type = other DNA
cctttgaatgccctccatgaataaaat

SEQ ID NO: 325 - DNA, 29 bp, synthetic construct
  misc_feature 1..29: note = Primer
  source 1..29: mol_type = other DNA
gcatatagaaaagatagaagttcgaaaga

SEQ ID NO: 326 - DNA, 27 bp, synthetic construct
  misc_feature 1..27: note = Primer
  source 1..27: mol_type = other DNA
tatggctagacggtaaacaaaatacag

SEQ ID NO: 327 - DNA, 26 bp, synthetic construct
  misc_feature 1..26: note = Primer
  source 1..26: mol_type = other DNA
ctctgaaccttcccatcaaaaacatc

SEQ ID NO: 328 - DNA, 25 bp, synthetic construct
  misc_feature 1..25: note = Primer
  source 1..25: mol_type = other DNA
ttactgttmgggtatttgaagatgg

SEQ ID NO: 329 - DNA, 21 bp, synthetic construct
  misc_feature 1..21: note = Primer
  source 1..21: mol_type = other DNA
ccgtttcataaggygagttgt

SEQ ID NO: 330 - DNA, 20 bp, synthetic construct
  misc_feature 1..20: note = Primer
  source 1..20: mol_type = other DNA
atgtcagagggatagatcca

SEQ ID NO: 331 - DNA, 23 bp, synthetic construct
  misc_feature 1..23: note = Primer
  source 1..23: mol_type = other DNA
tatagctactgtcaccagacaat

SEQ ID NO: 332 - DNA, 22 bp, synthetic construct
  misc_feature 1..22: note = Primer
  source 1..22: mol_type = other DNA
agttctgcgttttgtcactgtc

SEQ ID NO: 333 - DNA, 19 bp, synthetic construct
  misc_feature 1..19: note = Primer
  source 1..19: mol_type = other DNA
cggaagcacattgctgatt

SEQ ID NO: 334 - DNA, 26 bp, synthetic construct
  misc_feature 1..26: note = Primer
  source 1..26: mol_type = other DNA
gatacattaagacgcctaaaggatgc

SEQ ID NO: 335 - DNA, 23 bp, synthetic construct
  misc_feature 1..23: note = Primer
  source 1..23: mol_type = other DNA
ccttttgaccaattcggacaact

SEQ ID NO: 336 - DNA, 26 bp, synthetic construct
  misc_feature 1..26: note = Primer
  source 1..26: mol_type = other DNA
tggaataatcatcatcattacagcca

SEQ ID NO: 337 - DNA, 26 bp, synthetic construct
  misc_feature 1..26: note = Primer
  source 1..26: mol_type = other DNA
gagtcatatcacgatcttattctggc

SEQ ID NO: 338 - DNA, 21 bp, synthetic construct
  misc_feature 1..21: note = Primer
  source 1..21: mol_type = other DNA
taccagtctgcgtctgattcc

SEQ ID NO: 339 - DNA, 21 bp, synthetic construct
  misc_feature 1..21: note = Primer
  source 1..21: mol_type = other DNA
acgttgcgctcattacttctg

SEQ ID NO: 340 - DNA, 23 bp, synthetic construct
  misc_feature 1..23: note = Primer
  source 1..23: mol_type = other DNA
tgagttacctgaatcactggaag

SEQ ID NO: 341 - DNA, 21 bp, synthetic construct
  misc_feature 1..21: note = Primer
  source 1..21: mol_type = other DNA
tcgaggatgatagtgcaggtc

SEQ ID NO: 342 - DNA, 21 bp, synthetic construct
  misc_feature 1..21: note = Primer
  source 1..21: mol_type = other DNA
ctgcgttaggtggaataccat

SEQ ID NO: 343 - DNA, 24 bp, synthetic construct
  misc_feature 1..24: note = Primer
  source 1..24: mol_type = other DNA
ctgggtctcctcattacaagtatc

SEQ ID NO: 344 - DNA, 18 bp, synthetic construct
  misc_feature 1..18: note = Primer
  source 1..18: mol_type = other DNA
gttccagcctgccatctg

SEQ ID NO: 345 - DNA, 18 bp, synthetic construct
  misc_feature 1..18: note = Primer
  source 1..18: mol_type = other DNA
tcgccagcaacacttcag

SEQ ID NO: 346 - DNA, 18 bp, synthetic construct
  misc_feature 1..18: note = Primer
  source 1..18: mol_type = other DNA
aagcacgctggtggttac

SEQ ID NO: 347 - DNA, 19 bp, synthetic construct
  misc_feature 1..19: note = Primer
  source 1..19: mol_type = other DNA
ctggatggtgttggtggaa

SEQ ID NO: 348 - DNA, 20 bp, synthetic construct
  misc_feature 1..20: note = Primer
  source 1..20: mol_type = other DNA
cgcgagygctttctatcttg

SEQ ID NO: 349 - DNA, 20 bp, synthetic construct
  misc_feature 1..20: note = Primer
  source 1..20: mol_type = other DNA
gagasccactggttccagaa

SEQ ID NO: 350 - DNA, 43 bp, synthetic construct
  misc_feature 1..43: note = Primer
  source 1..43: mol_type = other DNA
acccaactgaatggagcgggcggacgaaaacccttgagcacag

SEQ ID NO: 351 - DNA, 47 bp, synthetic construct
  misc_feature 1..47: note = Primer
  source 1..47: mol_type = other DNA
acgcacttgacttgtcttcgccgggatgccttacctagacgcaatga

SEQ ID NO: 352 - DNA, 45 bp, synthetic construct
  misc_feature 1..45: note = Primer
  source 1..45: mol_type = other DNA
acccaactgaatggagcgcggcagccgttgaggcaaaagtgatac

SEQ ID NO: 353 - DNA, 48 bp, synthetic construct
  misc_feature 1..48: note = Primer
  source 1..48: mol_type = other DNA
acgcacttgacttgtcttccgagttccgtccggttaagcgtgacagtc

SEQ ID NO: 354 - DNA, 24 bp, synthetic construct
  misc_feature 1..24: note = Primer
  source 1..24: mol_type = other DNA
agaggaggagatagagtaggagat

SEQ ID NO: 355 - DNA, 25 bp, synthetic construct
  misc_feature 1..25: note = Primer
  source 1..25: mol_type = other DNA
taccagccagtatgataagaagaga

SEQ ID NO: 356 - DNA, 21 bp, synthetic construct
  misc_feature 1..21: note = Primer
  source 1..21: mol_type = other DNA
gcacgttgatgacttctgaca

SEQ ID NO: 357 - DNA, 23 bp, synthetic construct
  misc_feature 1..23: note = Primer
  source 1..23: mol_type = other DNA
gcccacaaacaatccaaccttac

SEQ ID NO: 358 - DNA, 24 bp, synthetic construct
  misc_feature 1..24: note = Primer
  source 1..24: mol_type = other DNA
tgcccataacacatttgacacttt

SEQ ID NO: 359 - DNA, 20 bp, synthetic construct
  misc_feature 1..20: note = Primer
  source 1..20: mol_type = other DNA
ttcggccacagctaaactcg

SEQ ID NO: 360 - DNA, 24 bp, synthetic construct
  misc_feature 1..24: note = Primer
  source 1..24: mol_type = other DNA
accttatacggaacatagcagacg

SEQ ID NO: 361 - DNA, 21 bp, synthetic construct
  misc_feature 1..21: note = Primer
  source 1..21: mol_type = other DNA
tcgatgcgcttctatcacttc

SEQ ID NO: 362 - DNA, 20 bp, synthetic construct
  misc_feature 1..20: note = Primer
  source 1..20: mol_type = other DNA
cgccaaatgactcgcattgt

SEQ ID NO: 363 - DNA, 22 bp, synthetic construct
  misc_feature 1..22: note = Primer
  source 1..22: mol_type = other DNA
gcatgtgcctttccgaartaaa

SEQ ID NO: 364 - DNA, 17 bp, synthetic construct
  misc_feature 1..17: note = Primer
  source 1..17: mol_type = other DNA
gcgcaacagggaagcaa

SEQ ID NO: 365 - DNA, 23 bp, synthetic construct
  misc_feature 1..23: note = Primer
  source 1..23: mol_type = other DNA
tgcggatgtcctatgtctgaaag

SEQ ID NO: 366 - DNA, 22 bp, synthetic construct
  misc_feature 1..22: note = Primer
  source 1..22: mol_type = other DNA
catgaccgccactataaccaga

SEQ ID NO: 367 - DNA, 22 bp, synthetic construct
  misc_feature 1..22: note = Primer
  source 1..22: mol_type = other DNA
atgcaacattagcaggaggatg

SEQ ID NO: 368 - DNA, 16 bp, synthetic construct
  misc_feature 1..16: note = Primer
  source 1..16: mol_type = other DNA
ctggcgctctccagca

SEQ ID NO: 369 - DNA, 25 bp, synthetic construct
  misc_feature 1..25: note = Primer
  source 1..25: mol_type = other DNA
ttgcaattagtgtgttaggtggtaa

SEQ ID NO: 370 - DNA, 20 bp, synthetic construct
  misc_feature 1..20: note = Primer
  source 1..20: mol_type = other DNA
gacaccatgcgttttgcttc

SEQ ID NO: 371 - DNA, 20 bp, synthetic construct
  misc_feature 1..20: note = Primer
  source 1..20: mol_type = other DNA
tcgtaccggcaacaattgac

SEQ ID NO: 372 - DNA, 20 bp, synthetic construct
  misc_feature 1..20: note = Primer
  source 1..20: mol_type = other DNA
gtggcgatttcacgctgtta

SEQ ID NO: 373 - DNA, 20 bp, synthetic construct
  misc_feature 1..20: note = Primer
  source 1..20: mol_type = other DNA
tatccagcacgttccaggtg

SEQ ID NO: 374 - DNA, 20 bp, synthetic construct
  misc_feature 1..20: note = Primer
  source 1..20: mol_type = other DNA
aaaaccgcgccgcgttacct

SEQ ID NO: 375 - DNA, 20 bp, synthetic construct
  misc_feature 1..20: note = Primer
  source 1..20: mol_type = other DNA
ccagaaatcgcgcccgcatt

SEQ ID NO: 376 - DNA, 20 bp, synthetic construct
  misc_feature 1..20: note = Primer
  source 1..20: mol_type = other DNA
tccagcaggtgctggatcgt

SEQ ID NO: 377 - DNA, 22 bp, synthetic construct
  misc_feature 1..22: note = Primer
  source 1..22: mol_type = other DNA
gcgaaatttttcgccgtactgt

SEQ ID NO: 378 - DNA, 24 bp, synthetic construct
  misc_feature 1..24: note = Primer
  source 1..24: mol_type = other DNA
cattacggcaaagtgtgggtcaat

SEQ ID NO: 379 - DNA, 24 bp, synthetic construct
  misc_feature 1..24: note = Primer
  source 1..24: mol_type = other DNA
ccatcagcacgttatcgaatcctt

SEQ ID NO: 380 - DNA, 23 bp, synthetic construct
  misc_feature 1..23: note = Primer
  source 1..23: mol_type = other DNA
cgtatcachgtttgtgtgaacaa

SEQ ID NO: 381 - DNA, 22 bp, synthetic construct
  misc_feature 1..22: note = Primer
  source 1..22: mol_type = other DNA
ggattcacyacttgcaaagtcc

SEQ ID NO: 382 - DNA, 20 bp, synthetic construct
  misc_feature 1..20: note = Prmer
  source 1..20: mol_type = other DNA
ataccgacgacgccgatctg

SEQ ID NO: 383 - DNA, 20 bp, synthetic construct
  misc_feature 1..20: note = Primer
  source 1..20: mol_type = other DNA
ggatcatttatgctggtacg

SEQ ID NO: 384 - DNA, 20 bp, synthetic construct
  misc_feature 1..20: note = Primer
  source 1..20: mol_type = other DNA
ataccgacgacgccgatctg

SEQ ID NO: 385 - DNA, 20 bp, synthetic construct
  misc_feature 1..20: note = Primer
  source 1..20: mol_type = other DNA
tgctattcattatgcgcagc

SEQ ID NO: 386 - DNA, 20 bp, synthetic construct
  misc_feature 1..20: note = Primer
  source 1..20: mol_type = other DNA
ggcgaaatggcwgagaacca

SEQ ID NO: 387 - DNA, 20 bp, synthetic construct
  misc_feature 1..20: note = Primer
  source 1..20: mol_type = other DNA
gagtcttcgaagttgtaacc

SEQ ID NO: 388 - DNA, 22 bp, synthetic construct
  misc_feature 1..22: note = Primer
  source 1..22: mol_type = other DNA
tgaaatatgactccactcacgg

SEQ ID NO: 389 - DNA, 24 bp, synthetic construct
  misc_feature 1..24: note = Primer
  source 1..24: mol_type = other DNA
cttcagaagcggctttgatggctt

SEQ ID NO: 390 - DNA, 21 bp, synthetic construct
  misc_feature 1..21: note = Primer
  source 1..21: mol_type = other DNA
cccaactcgcttcaggttcag

SEQ ID NO: 391 - DNA, 20 bp, synthetic construct
  misc_feature 1..20: note = Primer
  source 1..20: mol_type = other DNA
ccgtttttccccagcagcag

SEQ ID NO: 392 - DNA, 26 bp, synthetic construct
  misc_feature 1..26: note = Primer
  source 1..26: mol_type = other DNA
gagaaaaacctgcctgtactgctggc

SEQ ID NO: 393 - DNA, 25 bp, synthetic construct
  misc_feature 1..25: note = Primer
  source 1..25: mol_type = other DNA
cgcgccacgctttatagcggttaat

SEQ ID NO: 394 - DNA, 26 bp, synthetic construct
  misc_feature 1..26: note = Primer
  source 1..26: mol_type = other DNA
acctaccgcaacaccgacttcttcgg

SEQ ID NO: 395 - DNA, 21 bp, synthetic construct
  misc_feature 1..21: note = Primer
  source 1..21: mol_type = other DNA
tgatcagaactggtaggtgat

SEQ ID NO: 396 - DNA, 21 bp, synthetic construct
  misc_feature 1..21: note = Primer
  source 1..21: mol_type = other DNA
ctcgctgctggactatattcg

SEQ ID NO: 397 - DNA, 21 bp, synthetic construct
  misc_feature 1..21: note = Primer
  source 1..21: mol_type = other DNA
cgctttcagctcaagaacttc

SEQ ID NO: 398 - DNA, 24 bp, synthetic construct
  misc_feature 1..24: note = Primer
  source 1..24: mol_type = other DNA
ctttatacctcggtacatcaggtt

SEQ ID NO: 399 - DNA, 21 bp, synthetic construct
  misc_feature 1..21: note = Primer
  source 1..21: mol_type = other DNA
attcgccggctgrgcrgagag

SEQ ID NO: 400 - DNA, 17 bp, synthetic construct
  misc_feature 1..17: note = Primer
  source 1..17: mol_type = other DNA
atggtggtgcgccagtg

SEQ ID NO: 401 - DNA, 18 bp, synthetic construct
  misc_feature 1..18: note = Primer
  source 1..18: mol_type = other DNA
gctgaccgagacgttgtc

SEQ ID NO: 402 - DNA, 23 bp, synthetic construct
  misc_feature 1..23: note = Primer
  source 1..23: mol_type = other DNA
acggcaggcgatttgatttaacg

SEQ ID NO: 403 - DNA, 22 bp, synthetic construct
  misc_feature 1..22: note = Primer
  source 1..22: mol_type = other DNA
agctgcgtgatcgagacctatc

SEQ ID NO: 404 - DNA, 20 bp, synthetic construct
  misc_feature 1..20: note = Primer
  source 1..20: mol_type = other DNA
tcatcatctgcactttccgc

SEQ ID NO: 405 - DNA, 20 bp, synthetic construct
  misc_feature 1..20: note = Primer
  source 1..20: mol_type = other DNA
ccagatcagcgcgaacttca

SEQ ID NO: 406 - DNA, 20 bp, synthetic construct
  misc_feature 1..20: note = Primer
  source 1..20: mol_type = other DNA
tcacaggtcgccagcgcttc

SEQ ID NO: 407 - DNA, 20 bp, synthetic construct
  misc_feature 1..20: note = Primer
  source 1..20: mol_type = other DNA
tcccggcagataagctgtgg

SEQ ID NO: 408 - DNA, 20 bp, synthetic construct
  misc_feature 1..20: note = Primer
  source 1..20: mol_type = other DNA
tcggcgacacggatgacggc

SEQ ID NO: 409 - DNA, 20 bp, synthetic construct
  misc_feature 1..20: note = Primer
  source 1..20: mol_type = other DNA
gtccatgtaggcgttcaggg

SEQ ID NO: 410 - DNA, 29 bp, synthetic construct
  misc_feature 1..29: note = Primer
  source 1..29: mol_type = other DNA
atggaaagtaaagtagttgttccggcaca

SEQ ID NO: 411 - DNA, 19 bp, synthetic construct
  misc_feature 1..19: note = Primer
  source 1..19: mol_type = other DNA
ggacgcagcaggatctgtt

SEQ ID NO: 412 - DNA, 20 bp, synthetic construct
  misc_feature 1..20: note = Primer
  source 1..20: mol_type = other DNA
agcgcgttctgttcaaatgc

SEQ ID NO: 413 - DNA, 21 bp, synthetic construct
  misc_feature 1..21: note = Primer
  source 1..21: mol_type = other DNA
caggttcagaactctctctgt

SEQ ID NO: 414 - DNA, 20 bp, synthetic construct
  misc_feature 1..20: note = Primer
  source 1..20: mol_type = other DNA
tcggtaacggtgttgtgctg

SEQ ID NO: 415 - DNA, 20 bp, synthetic construct
  misc_feature 1..20: note = Primer
  source 1..20: mol_type = other DNA
catacggtaagccacgcaga

SEQ ID NO: 416 - DNA, 20 bp, synthetic construct
  misc_feature 1..20: note = Primer
  source 1..20: mol_type = other DNA
acctttgtagctgtaccacg

SEQ ID NO: 417 - DNA, 21 bp, synthetic construct
  misc_feature 1..21: note = Primer
  source 1..21: mol_type = other DNA
agcgtgaaggtaaaacctgtg

SEQ ID NO: 418 - DNA, 23 bp, synthetic construct
  misc_feature 1..23: note = Primer
  source 1..23: mol_type = other DNA
ttgattcaccagcgcgtattgtc

SEQ ID NO: 419 - DNA, 21 bp, synthetic construct
  misc_feature 1..21: note = Primer
  source 1..21: mol_type = other DNA
aggtatctgcttcaatcagcg

SEQ ID NO: 420 - DNA, 23 bp, synthetic construct
  misc_feature 1..23: note = Primer
  source 1..23: mol_type = other DNA
atcggaaatcctatttcacattc

SEQ ID NO: 421 - DNA, 23 bp, synthetic construct
  misc_feature 1..23: note = Primer
  source 1..23: mol_type = other DNA
ggtgttgtattaataacgatatc

SEQ ID NO: 422 - DNA, 22 bp, synthetic construct
  misc_feature 1..22: note = Primer
  source 1..22: mol_type = other DNA
ctaggaactgcaatcttaatcc

SEQ ID NO: 423 - DNA, 23 bp, synthetic construct
  misc_feature 1..23: note = Primer
  source 1..23: mol_type = other DNA
tggtaaaatcgcatgtccaattc

SEQ ID NO: 424 - DNA, 20 bp, synthetic construct
  misc_feature 1..20: note = Primer
  source 1..20: mol_type = other DNA
atcgttttatcgggaccatc

SEQ ID NO: 425 - DNA, 23 bp, synthetic construct
  misc_feature 1..23: note = Primer
  source 1..23: mol_type = other DNA
tcattaactacaacgtaatcgta

SEQ ID NO: 426 - DNA, 23 bp, synthetic construct
  misc_feature 1..23: note = Primer
  source 1..23: mol_type = other DNA
gttaaaatcgtattacctgaagg

SEQ ID NO: 427 - DNA, 23 bp, synthetic construct
  misc_feature 1..23: note = Primer
  source 1..23: mol_type = other DNA
gacccttttgttgaaaagcttaa

SEQ ID NO: 428 - DNA, 23 bp, synthetic construct
  misc_feature 1..23: note = Primer
  source 1..23: mol_type = other DNA
tcgttcattctgaacgtcgtgaa

SEQ ID NO: 429 - DNA, 23 bp, synthetic construct
  misc_feature 1..23: note = Primer
  source 1..23: mol_type = other DNA
tttgcaccttctaacaattgtac

SEQ ID NO: 430 - DNA, 23 bp, synthetic construct
  misc_feature 1..23: note = Primer
  source 1..23: mol_type = other DNA
cagcatacaggacacctattggc

SEQ ID NO: 431 - DNA, 23 bp, synthetic construct
  misc_feature 1..23: note = Primer
  source 1..23: mol_type = other DNA
cgttgaggaatcgatactggaac